European Patent Specification EP 3 460 065 B1, published August 23, 2023. Title: CELL TRANSFECTION METHOD. Applicant: Commonweath Scientific and Industrial Research Organisation MAT Malta Advanced Technologies Limited. Application EP. The sequence listing filed with the application follows.

SEQUENCE LISTING (10 sequences)

SEQ ID NO: 1 - DNA, 4090 bp, Artificial Sequence
  EGFP expression construct flanked by Tol2 sequences
cagaggtgtaaagtacttgagtaattttacttgattactgtacttaagtattatttttggggatttttactttacttgagtacaattaaaaatcaatacttttacttttacttaattacatttttttagaaaaaaaagtactttttactccttacaattttatttacagtcaaaaagtacttattttttggagatcacttcattctattttcccttgctattaccaaaccaattgaattgcgctgatgcccagtttaatttaaatgttatttattctgcctatgaaaatcgttttcacattatatgaaattggtcagacatgttcattggtcctttggaagtgacgtcatgtcacatctattaccacaatgcacagcaccttgacctggaaattagggaaattataacagtcaatcagtggaagaaaatggaggaagtatgtgattcatcagcagctgcgagcagcacagtccaaaatcagccacaggatcaagagcacccgtggccgtatcttcgcagatcgacattgattattgactagttattaatagtaatcaattacggggtcattagttcatagcccatatatggagttccgcgttacataacttacggtaaatggcccgcctggctgaccgcccaacgacccccgcccattgacgtcaataatgacgtatgttcccatagtaacgccaatagggactttccattgacgtcaatgggtggagtatttacggtaaactgcccacttggcagtacatcaagtgtatcatatgccaagtacgccccctattgacgtcaatgacggtaaatggcccgcctggcattatgcccagtacatgaccttatgggactttcctacttggcagtacatctacgtattagtcatcgctattaccatgggtcgaggtgagccccacgttctgcttcactctccccatctcccccccctccccacccccaattttgtatttatttattttttaattattttgtgcagcgatgggggcggggggggggggggcgcgcgccaggcggggcggggcggggcgaggggcggggcggggcgaggcggagaggtgcggcggcagccaatcagagcggcgcgctccgaaagtttccttttatggcgaggcggcggcggcggcggccctataaaaagcgaagcgcgcggcgggcgggagtcgctgcgttgccttcgccccgtgccccgctccgcgccgcctcgcgccgcccgccccggctctgactgaccgcgttactcccacaggtgagcgggcgggacggcccttctcctccgggctgtaattagcgcttggtttaatgacggctcgtttcttttctgtggctgcgtgaaagccttaaagggctccgggagggccctttgtgcgggggggagcggctcggggggtgcgtgcgtgtgtgtgtgcgtggggagcgccgcgtgcggcccgcgctgcccggcggctgtgagcgctgcgggcgcggcgcggggctttgtgcgctccgcgtgtgcgcgaggggagcgcggccgggggcggtgccccgcggtgcgggggggctgcgaggggaacaaaggctgcgtgcggggtgtgtgcgtgggggggtgagcagggggtgtgggcgcggcggtcgggctgtaacccccccctgcacccccctccccgagttgctgagcacggcccggcttcgggtgcggggctccgtgcggggcgtggcgcggggctcgccgtgccgggcggggggtggcggcaggtgggggtgccgggcggggcggggccgcctcgggccggggagggctcgggggaggggcgcggcggccccggagcgccggcggctgtcgaggcgcggcgagccgcagccattgccttttatggtaatcgtgcgagagggcgcagggacttcctttgtcccaaatctggcggagccgaaatctgggaggcgccgccgcaccccctctagcgggcgcggggcgaagcggtgcggcgccggcaggaaggaaatgggcggggagggccttcgtgcgtcgccgcgccgccgtccccttctccctctccagcctcggggctgtccgcggggggacggctgccttcgggggggacggggcagggcggggttcggcttctggcgtgtgaccggcggctctagagcctctgctaaccatgttcatgccttcttctttttcctacagctcctgggcaacgtgctggttattgtgctgtctcatcattttggcaaagaattgtaccaccatggtgagcaagggcgaggagctgttcaccggggtggtgcccatcctggtcgagctggacggcgacgtaaacggccacaagttcagcgtgtccggcgagggcgagggcgatgccacctacggcaagctgaccctgaagttcatctgcaccaccggcaagctgcccgtgccctggcccacactagtgaccaccttcgcttacggcgtgcagtgcttcagccgctaccccgaccacatgaagcagcacgacttcttcaagtccgccatgcccgaaggctacgtccaggagcgcaccatcttcttcaaggacgacggcaactacaagacccgcgccgaggtgaagttcgagggcgacaccctggtgaaccgcatcgagctgaagggcatcgacttcaaggaggacggcaacatcctggggcacaagctggagtacaacttcaacagccacaacgtatacatcatggccgacaagcagaagaacggcatcaaggtgaacttcaagatccgccacaacatcgaggacggcagcgtgcagctcgccgaccactaccagcagaacacccccatcggcgacggccccgtgctgctgcccgacaaccactacctgagcacccagtccgccctgagcaaagaccccaacgagaagcgcgatcacatggtcctgctggagttcgtgaccgccgccgggatcactcacggcatggacgagctgtacaagtagggcggctcgaggatatcaggatcaattcactcctcaggtgcaggctgcctatcagaaggtggtggctggtgtggccaatgccctggctcacaaataccactgagatctttttccctctgccaaaaattatggggacatcatgaagccccttgagcatctgacttctggctaataaaggaaatttattttcattgcaatagtgtgttggaattttttgtgtctctcactcggaaggacatatgggagggcaaatcatttaaaacatcagaatgagtatttggtttagagtttggcaacatatgcccatatgctggctgccatgaacaaaggttggctataaagaggtcatcagtatatgaaacagccccctgctgtccattccttattccatagaaaagccttgacttgaggttagattttttttatattttgttttgtgttatttttttctttaacatccctaaaattttccttacatgttttactagccagatttttcctcctctcctgactactcccagtcatagctgtccctcttctcttatggagatccctcgacctgcagcccaagctcgagggcccatctggcctgtgtttcagacaccagggagtctctgctcacgtttcctgctatttgcagcctctctatcaagactaatacacctcttcccgcatcggctgcctgtgagaggcttttcagcactgcaggattgcttttcagccccaaaagagctaggcttgacactaacaattttgagaatcagcttctactgaagttaaatctgaggttttacaactttgagtagcgtgtactggcattagattgtctgtcttatagtttgataattaaatacaaacagttctaaagcaggataaaaccttgtatgcatttcatttaatgttttttgagattaaaagcttaaacaagaatctctagttttctttcttgcttttacttttacttccttaatactcaagtacaattttaatggagtacttttttacttttactcaagtaagattctagccagatacttttacttttaattgagtaaaattttccctaagtacttgtactttcacttgagtaaaatttttgagtactttttacacctctg

SEQ ID NO: 2 - protein, 706 aa, Artificial Sequence
  Sequence encoding Tol2 transposase
MFMPSSFSYSSWATCWLLCCLIILAKNSSRSSHIYYHNAQHLDLEIREIITVNQWKKMEEVCDSSAAASSTVQNQPQDQEHPWPYLREFFSLSGVNKDSFKMKCVLCLPLNKEISAFKSSPSNLRKHIERMHPNYLKNYSKLTAQKRKIGTSTHASSSKQLKVDSVFPVKHVSPVTVNKAILRYIIQGLHPFSTVDLPSFKELISTLQPGISVITRPTLRSKIAEAALIMKQKVTAAMSEVEWIATTTDCWTARRKSFIGVTAHWINPGSLERHSAALACKRLMGSHTFEVLASAMNDIHSEYEIRDKVVCTTTDSGSNFMKAFRVFGVENNDIETEARRCESDDTDSEGCGEGSDGVEFQDASRVLDQDDGFEFQLPKHQKCACHLLNLVSSVDAQKALSNEHYKKLYRSVFGKCQALWNKSSRSALAAEAVESESRLQLLRPNQTRWNSTFMAVDRILQICKEAGEGALRNICTSLEVPMFNPAEMLFLTEWANTMRPVAKVLDILQAETNTQLGWLLPSVHQLSLKLQRLHHSLRYCDPLVDALQQGIQTRFKHMFEDPEIIAAAILLPKFRTSWTNDETIIKRGMDYIRVHLEPLDHKKELANSSSDDEDFFASLKPTTHEASKELDGYLACVSDTRESLLTFPAICSLSIKTNTPLPASAACERLFSTAGLLFSPKRARLDTNNFENQLLLKLNLRFYNFE

SEQ ID NO: 3 - DNA, 20 bp, Artificial Sequence
  Screen 7 oligonucleotide primer
gtgactcagactcctgttag

SEQ ID NO: 4 - DNA, 20 bp, Artificial Sequence
  Screen 6 oligonucleotide primer
tctgctgcttcacagtcttc

SEQ ID NO: 5 - DNA, 33 bp, Artificial Sequence
  miniTol2 forward oligonucleotide primer
cagtcaaaaagtacttattttttggagatcact

SEQ ID NO: 6 - DNA, 21 bp, Artificial Sequence
  miniTol2 Reverse oligonucleotide primer
gggcatcagcgcaattcaatt

SEQ ID NO: 7 - DNA, 17 bp, Artificial Sequence
  miniTol2 detection probe
atagcaagggaaaatag

SEQ ID NO: 8 - DNA, 21 bp, Artificial Sequence
  Genomic control region forward primer
gatgggaaaaccctgaacctc

SEQ ID NO: 9 - DNA, 26 bp, Artificial Sequence
  Genomic region control reverse primer
caacctgctagagaagatgagaagag

SEQ ID NO: 10 - DNA, 15 bp, Artificial Sequence
  Genomic control region oligonucleotide probe
ctgcactgaatggac